European Patent Application EP 4 696 774 A1, published February 18, 2026. Title: O-phosphoserine sulfhydrylase variant and method for producing cysteine using the same. Applicant: CJ CheilJedang Corporation. The sequence listing filed with the application follows.

SEQUENCE LISTING (23 sequences)

SEQ ID NO: 1 - protein, 323 aa, unidentified
MTRYDSLLQALGNTPLVGLQNLSPRWDDEDGKPHVRLWAKLEDRNPTGSIKDRPALRMIEQAERDGLLQPGATILEPTSGNTGISLAMAALLKGYNMICVMPENTSIERRQILELYGARIIFSPAEGGSNTAVATAKELAAQNPSWVMLYQYGNPANSDAHYFGTGPELLADLPEITHFVAGLGTTGTLMGTGRFLREHVPGVQIVAAEPRYGEGVYALRNIDEGFIPELYDADVLTTRFSVGSFDAVRRTRELVTREGIFAGISTGAVLHAALGMAAKAVKAGERADIAFVVADAGWKYLSTGAYAGSLDDAEDALEGQLWA

SEQ ID NO: 2 - DNA, 972 bp, unidentified
  source 1..972: mol_type = genomic DNA
gtgacgcgctacgactccctgctgcaggccctgggcaacaccccgctggtgggcctgcagaacctgtcgccccggtgggacgacgaggacgggaaaccccacgtgcggctgtgggccaagctcgaggaccgcaacccgaccggttccatcaaggaccgccccgcgctgcggatgatcgaacaggccgagcgcgacgggctgctgcagcccggcgccacgatcctggaacccaccagcggcaacaccggcatctcgctggccatggcggccctgctcaagggctacaacatgatctgcgtgatgccggagaacacgtcgatcgaacggcgccagatcctcgagctctacggcgcgcgcatcatcttcagccccgccgagggcggctccaacaccgcggtcgcgaccgcgaaagagcttgccgcgcagaacccgtcgtgggtcatgctgtatcagtacggcaacccggccaacagcgatgcgcactacttcggcaccggccccgaactgctcgcggacctgcccgagatcacccacttcgtcgcggggctcggcaccaccgggaccctgatgggcaccggacgtttcctgcgcgagcacgttcccggcgtgcagatcgtggcggccgaaccgcgttacggcgagggcgtgtacgcactgcgcaacatcgacgagggcttcatccccgagttgtacgacgccgacgtgctcaccacccggttctcggtgggctcgttcgacgccgtgcgccgcacccgtgaactcgtcacgcgcgagggcatattcgcgggcatctcgaccggcgcggtgctgcacgccgcgctggggatggccgccaaggccgtcaaggccggtgagcgtgccgacatcgcgttcgtcgtcgccgacgccggatggaagtatctgtcgaccggcgcgtacgccggtagcctggatgacgccgaggacgcgctggaagggcagctatgggcatga

SEQ ID NO: 3 - protein, 318 aa, synthetic construct
MTRYDSLLQALGNTPLVGLQNLSPRWDDEDGKPHVRLWAKLEDRNPTGSIKDRPALRMIEQAERDGLLQPGATILEATSGNTGISLAMAALLKGYNMICVMPENTSIERRQILELYGARIIFSPAEGGSNTAVATAKELAAQNPSWVMLYQYGNPANSDAHYFGTGPELLADLPEITHFVAGLGTTGTLMGTGRFLREHVPGVQIVAAEPRYGEGVYALRNIDEGFIPELYDADVLTTRFSVGSFDAVRRTRELVTREGIFAGISTGAVLHAALGMAAKAVKAGERADIAFVVADAGWKYLSTGAYAGSLDDAEDALE

SEQ ID NO: 4 - DNA, 957 bp, synthetic construct
  source 1..957: mol_type = other DNA
gtgacgcgctacgactccctgctgcaggccctgggcaacaccccgctggtgggcctgcagaacctgtcgccccggtgggacgacgaggacgggaaaccccacgtgcggctgtgggccaagctcgaggaccgcaacccgaccggttccatcaaggaccgccccgcgctgcggatgatcgaacaggccgagcgcgacgggctgctgcagcccggcgccacgatcctggaagccaccagcggcaacaccggcatctcgctggccatggcggccctgctcaagggctacaacatgatctgcgtgatgccggagaacacgtcgatcgaacggcgccagatcctcgagctctacggcgcgcgcatcatcttcagccccgccgagggcggctccaacaccgcggtcgcgaccgcgaaagagcttgccgcgcagaacccgtcgtgggtcatgctgtatcagtacggcaacccggccaacagcgatgcgcactacttcggcaccggccccgaactgctcgcggacctgcccgagatcacccacttcgtcgcggggctcggcaccaccgggaccctgatgggcaccggacgtttcctgcgcgagcacgttcccggcgtgcagatcgtggcggccgaaccgcgttacggcgagggcgtgtacgcactgcgcaacatcgacgagggcttcatccccgagttgtacgacgccgacgtgctcaccacccggttctcggtgggctcgttcgacgccgtgcgccgcacccgtgaactcgtcacgcgcgagggcatattcgcgggcatctcgaccggcgcggtgctgcacgccgcgctggggatggccgccaaggccgtcaaggccggtgagcgtgccgacatcgcgttcgtcgtcgccgacgccggatggaagtatctgtcgaccggcgcgtacgccggtagcctggatgacgccgaggacgcgctggaataa

SEQ ID NO: 5 - protein, 318 aa, synthetic construct
MTRYDSLLQALGNTPLVGLQNLSPRWDDEDGKPHVRLWAKLEDRNPTGSIKDRPALRMIEQAERDGLLQPGATILEATSGNTGISLAMAALLKGYNMICVMPENTSIERRQILELYGARIIFSPAEGGSNTAVATAKELAAQNPSWVMLYQYGNPANSDAHYFGTGPELLADLPEITHFVAGLGTTGTLMGTGRFLREHVPGVQIVAAEPRYGEGVYGLRNIDEGFIPELYDADVLTTRFSVGSFDAVRRTRELVTREGIFAGISTGAVLHAALGMAAKAVKAGERADIAFVVADAGWKYLSTGAYAGSLDDAEDALE

SEQ ID NO: 6 - DNA, 957 bp, synthetic construct
  source 1..957: mol_type = other DNA
gtgacgcgctacgactccctgctgcaggccctgggcaacaccccgctggtgggcctgcagaacctgtcgccccggtgggacgacgaggacgggaaaccccacgtgcggctgtgggccaagctcgaggaccgcaacccgaccggttccatcaaggaccgccccgcgctgcggatgatcgaacaggccgagcgcgacgggctgctgcagcccggcgccacgatcctggaagccaccagcggcaacaccggcatctcgctggccatggcggccctgctcaagggctacaacatgatctgcgtgatgccggagaacacgtcgatcgaacggcgccagatcctcgagctctacggcgcgcgcatcatcttcagccccgccgagggcggctccaacaccgcggtcgcgaccgcgaaagagcttgccgcgcagaacccgtcgtgggtcatgctgtatcagtacggcaacccggccaacagcgatgcgcactacttcggcaccggccccgaactgctcgcggacctgcccgagatcacccacttcgtcgcggggctcggcaccaccgggaccctgatgggcaccggacgtttcctgcgcgagcacgttcccggcgtgcagatcgtggcggccgaaccgcgttacggcgagggcgtgtacggcctgcgcaacatcgacgagggcttcatccccgagttgtacgacgccgacgtgctcaccacccggttctcggtgggctcgttcgacgccgtgcgccgcacccgtgaactcgtcacgcgcgagggcatattcgcgggcatctcgaccggcgcggtgctgcacgccgcgctggggatggccgccaaggccgtcaaggccggtgagcgtgccgacatcgcgttcgtcgtcgccgacgccggatggaagtatctgtcgaccggcgcgtacgccggtagcctggatgacgccgaggacgcgctggaataa

SEQ ID NO: 7 - protein, 318 aa, synthetic construct
MTRYDSLLQALGNTPLVGLQNLSPRWDDEDGKPHVRLWAKLEDRNPTGSIKDRPVLRMIEQAERDGLLQPGATILEATSGNTGISLAMAALLKGYNMICVMPENTSIERRQILELYGARIIFSPAEGGSNTAVATAKELAAQNPSWVMLYQYGNPANSDAHYFGTGPELLADLPEITHFVAGLGTTGTLMGTGRFLREHVPGVQIVAAEPRYGEGVYGLRNIDEGFIPELYDADVLTTRFSVGSFDAVRRTRELVTREGIFAGISTGAVLHAALGMAAKAVKAGERADIAFVVADAGWKYLSTGAYAGSLDDAEDALE

SEQ ID NO: 8 - DNA, 957 bp, synthetic construct
  source 1..957: mol_type = other DNA
gtgacgcgctacgactccctgctgcaggccctgggcaacaccccgctggtgggcctgcagaacctgtcgccccggtgggacgacgaggacgggaaaccccacgtgcggctgtgggccaagctcgaggaccgcaacccgaccggttccatcaaggaccgccccgtgctgcggatgatcgaacaggccgagcgcgacgggctgctgcagcccggcgccacgatcctggaagccaccagcggcaacaccggcatctcgctggccatggcggccctgctcaagggctacaacatgatctgcgtgatgccggagaacacgtcgatcgaacggcgccagatcctcgagctctacggcgcgcgcatcatcttcagccccgccgagggcggctccaacaccgcggtcgcgaccgcgaaagagcttgccgcgcagaacccgtcgtgggtcatgctgtatcagtacggcaacccggccaacagcgatgcgcactacttcggcaccggccccgaactgctcgcggacctgcccgagatcacccacttcgtcgcggggctcggcaccaccgggaccctgatgggcaccggacgtttcctgcgcgagcacgttcccggcgtgcagatcgtggcggccgaaccgcgttacggcgagggcgtgtacggcctgcgcaacatcgacgagggcttcatccccgagttgtacgacgccgacgtgctcaccacccggttctcggtgggctcgttcgacgccgtgcgccgcacccgtgaactcgtcacgcgcgagggcatattcgcgggcatctcgaccggcgcggtgctgcacgccgcgctggggatggccgccaaggccgtcaaggccggtgagcgtgccgacatcgcgttcgtcgtcgccgacgccggatggaagtatctgtcgaccggcgcgtacgccggtagcctggatgacgccgaggacgcgctggaataa

SEQ ID NO: 9 - protein, 318 aa, synthetic construct
MTRYDSPLQALGNTPLVGLQNLSPRWDDEDGKPHVRLWAKLEDRNPTGSIKDRPALRMIEQAERDGLLQPGATILEATSGNTGISLAMAALLKGYNMICVMPENTSIERRQILELYGARIIFSPAEGGSNTAVATAKELAAQNPSWVMLYQYGNPANSDAHYFGTGPELLADLPEITHFVAGLGTTGTLMGTGRFLREHVPGVQIVAAEPRYGEGVYGLRNIDEGFIPELYDADVLTTRFSVGSFDAVRRTRELVTREGIFAGISTGAVLHAALGMAAKAVKAGERADIAFVVADAGWKYLSTGAYAGSLDDAEDALE

SEQ ID NO: 10 - DNA, 957 bp, synthetic construct
  source 1..957: mol_type = other DNA
gtgacgcgctacgactccccgctgcaggccctgggcaacaccccgctggtgggcctgcagaacctgtcgccccggtgggacgacgaggacgggaaaccccacgtgcggctgtgggccaagctcgaggaccgcaacccgaccggttccatcaaggaccgccccgcgctgcggatgatcgaacaggccgagcgcgacgggctgctgcagcccggcgccacgatcctggaagccaccagcggcaacaccggcatctcgctggccatggcggccctgctcaagggctacaacatgatctgcgtgatgccggagaacacgtcgatcgaacggcgccagatcctcgagctctacggcgcgcgcatcatcttcagccccgccgagggcggctccaacaccgcggtcgcgaccgcgaaagagcttgccgcgcagaacccgtcgtgggtcatgctgtatcagtacggcaacccggccaacagcgatgcgcactacttcggcaccggccccgaactgctcgcggacctgcccgagatcacccacttcgtcgcggggctcggcaccaccgggaccctgatgggcaccggacgtttcctgcgcgagcacgttcccggcgtgcagatcgtggcggccgaaccgcgttacggcgagggcgtgtacggcctgcgcaacatcgacgagggcttcatccccgagttgtacgacgccgacgtgctcaccacccggttctcggtgggctcgttcgacgccgtgcgccgcacccgtgaactcgtcacgcgcgagggcatattcgcgggcatctcgaccggcgcggtgctgcacgccgcgctggggatggccgccaaggccgtcaaggccggtgagcgtgccgacatcgcgttcgtcgtcgccgacgccggatggaagtatctgtcgaccggcgcgtacgccggtagcctggatgacgccgaggacgcgctggaataa

SEQ ID NO: 11 - protein, 318 aa, synthetic construct
MTRYDSLLQALGNTPLVGLQNLSPRWDDEDGKPHVRLWAKLEDRNPTGSIKDRPALRMIEQAERDGLLQPGATILESTSGNTGISLAMAALLKGYNMICVMPENTSIERRQILELYGARIIFSPAEGGSNTAVATAKELAAQNPSWVMLYQYGNPANSDAHYFGTGPELLADLPEITHFVAGLGTTGTLMGTGRFLREHVPGVQIVAAEPRYGEGVYALRNIDEGFIPELYDADVLTTRFSVGSFDAVRRTRELVTREGIFAGISTGAVLHAALGMAAKAVKAGERADIAFVVADAGWKYLSTGAYAGSLDDAEDALE

SEQ ID NO: 12 - DNA, 957 bp, synthetic construct
  source 1..957: mol_type = other DNA
atgacgcgctacgactccctgctgcaggccctgggcaacaccccgctggtgggcctgcagaacctgtcgccccggtgggacgacgaggacgggaaaccccacgtgcggctgtgggccaagctcgaggaccgcaacccgaccggttccatcaaggaccgccccgcgctgcggatgatcgaacaggccgagcgcgacgggctgctgcagcccggcgccacgatcctggaatccaccagcggcaacaccggcatctcgctggccatggcggccctgctcaagggctacaacatgatctgcgtgatgccggagaacacgtcgatcgaacggcgccagatcctcgagctctacggcgcgcgcatcatcttcagccccgccgagggcggctccaacaccgcggtcgcgaccgcgaaagagcttgccgcgcagaacccgtcgtgggtcatgctgtatcagtacggcaacccggccaacagcgatgcgcactacttcggcaccggccccgaactgctcgcggacctgcccgagatcacccacttcgtcgcggggctcggcaccaccgggaccctgatgggcaccggacgtttcctgcgcgagcacgttcccggcgtgcagatcgtggcggccgaaccgcgttacggcgagggcgtgtacgcactgcgcaacatcgacgagggcttcatccccgagttgtacgacgccgacgtgctcaccacccggttctcggtgggctcgttcgacgccgtgcgccgcacccgtgaactcgtcacgcgcgagggcatattcgcgggcatctcgaccggcgcggtgttgcacgccgcgctggggatggccgccaaggccgtcaaggccggtgagcgtgccgacatcgcgttcgtcgtcgccgacgccggatggaagtatctgtcgaccggcgcgtacgccggtagcctggatgacgccgaggacgcgctggaataa

SEQ ID NO: 13 - protein, 318 aa, synthetic construct
MTRYDSLLQALGNTPLVGLQNLSPRWDDEDGKPHVRLWAKLEDRNPTGSIKDRPALRMIEQAERDGLLQPGATILEPTSGNTGISLAMAALLKGYNMICVMPENTSIERRQILELYGARIIFSPAEGGSNTAVATAKELAAQNPSWVMLYQYGNPANSDAHYFGTGPELLADLPEITHFVAGLGTTGTLMGTGRFLREHVPGVQIVAAEPRYGEGVYALRNIDEGFIPELYDADVLTTRFSVGSFDAVRRTRELVTREGIFAGISTGAVLHAALGMAAKAVKAGERADIAFVVADAGWKYLSTGAYAGSLDDAEDALE

SEQ ID NO: 14 - DNA, 957 bp, synthetic construct
  source 1..957: mol_type = other DNA
atgacgcgctacgactccctgctgcaggccctgggcaacaccccgctggtgggcctgcagaacctgtcgccccggtgggacgacgaggacgggaaaccccacgtgcggctgtgggccaagctcgaggaccgcaacccgaccggttccatcaaggaccgccccgcgctgcggatgatcgaacaggccgagcgcgacgggctgctgcagcccggcgccacgatcctggaacccaccagcggcaacaccggcatctcgctggccatggcggccctgctcaagggctacaacatgatctgcgtgatgccggagaacacgtcgatcgaacggcgccagatcctcgagctctacggcgcgcgcatcatcttcagccccgccgagggcggctccaacaccgcggtcgcgaccgcgaaagagcttgccgcgcagaacccgtcgtgggtcatgctgtatcagtacggcaacccggccaacagcgatgcgcactacttcggcaccggccccgaactgctcgcggacctgcccgagatcacccacttcgtcgcggggctcggcaccaccgggaccctgatgggcaccggacgtttcctgcgcgagcacgttcccggcgtgcagatcgtggcggccgaaccgcgttacggcgagggcgtgtacgcactgcgcaacatcgacgagggcttcatccccgagttgtacgacgccgacgtgctcaccacccggttctcggtgggctcgttcgacgccgtgcgccgcacccgtgaactcgtcacgcgcgagggcatattcgcgggcatctcgaccggcgcggtgttgcacgccgcgctggggatggccgccaaggccgtcaaggccggtgagcgtgccgacatcgcgttcgtcgtcgccgacgccggatggaagtatctgtcgaccggcgcgtacgccggtagcctggatgacgccgaggacgcgctggaataa

SEQ ID NO: 15 - DNA, 2686 bp, synthetic construct
  source 1..2686: mol_type = other DNA
gcgcccaatacgcaaaccgcctctccccgcgcgttggccgattcattaatgcagctggcacgacaggtttcccgactggaaagcgggcagtgagcgcaacgcaattaatgtgagttagctcactcattaggcaccccaggctttacactttatgcttccggctcgtatgttgtgtggaattgtgagcggataacaatttcacacaggaaacagctatgaccatgattacgccaagcttgcatgcctgcaggtcgactctagaggatccccgggtaccgagctcgaattcactggccgtcgttttacaacgtcgtgactgggaaaaccctggcgttacccaacttaatcgccttgcagcacatccccctttcgccagctggcgtaatagcgaagaggcccgcaccgatcgcccttcccaacagttgcgcagcctgaatggcgaatggcgcctgatgcggtattttctccttacgcatctgtgcggtatttcacaccgcatatggtgcactctcagtacaatctgctctgatgccgcatagttaagccagccccgacacccgccaacacccgctgacgcgccctgacgggcttgtctgctcccggcatccgcttacagacaagctgtgaccgtctccgggagctgcatgtgtcagaggttttcaccgtcatcaccgaaacgcgcgagacgaaagggcctcgtgatacgcctatttttataggttaatgtcatgataataatggtttcttagacgtcaggtggcacttttcggggaaatgtgcgcggaacccctatttgtttatttttctaaatacattcaaatatgtatccgctcatgagacaataaccctgataaatgcttcaataatattgaaaaaggaagagtatgagtattcaacatttccgtgtcgcccttattcccttttttgcggcattttgccttcctgtttttgctcacccagaaacgctggtgaaagtaaaagatgctgaagatcagttgggtgcacgagtgggttacatcgaactggatctcaacagcggtaagatccttgagagttttcgccccgaagaacgttttccaatgatgagcacttttaaagttctgctatgtggcgcggtattatcccgtattgacgccgggcaagagcaactcggtcgccgcatacactattctcagaatgacttggttgagtactcaccagtcacagaaaagcatcttacggatggcatgacagtaagagaattatgcagtgctgccataaccatgagtgataacactgcggccaacttacttctgacaacgatcggaggaccgaaggagctaaccgcttttttgcacaacatgggggatcatgtaactcgccttgatcgttgggaaccggagctgaatgaagccataccaaacgacgagcgtgacaccacgatgcctgtagcaatggcaacaacgttgcgcaaactattaactggcgaactacttactctagcttcccggcaacaattaatagactggatggaggcggataaagttgcaggaccacttctgcgctcggcccttccggctggctggtttattgctgataaatctggagccggtgagcgtgggtctcgcggtatcattgcagcactggggccagatggtaagccctcccgtatcgtagttatctacacgacggggagtcaggcaactatggatgaacgaaatagacagatcgctgagataggtgcctcactgattaagcattggtaactgtcagaccaagtttactcatatatactttagattgatttaaaacttcatttttaatttaaaaggatctaggtgaagatcctttttgataatctcatgaccaaaatcccttaacgtgagttttcgttccactgagcgtcagaccccgtagaaaagatcaaaggatcttcttgagatcctttttttctgcgcgtaatctgctgcttgcaaacaaaaaaaccaccgctaccagcggtggtttgtttgccggatcaagagctaccaactctttttccgaaggtaactggcttcagcagagcgcagataccaaatactgttcttctagtgtagccgtagttaggccaccacttcaagaactctgtagcaccgcctacatacctcgctctgctaatcctgttaccagtggctgctgccagtggcgataagtcgtgtcttaccgggttggactcaagacgatagttaccggataaggcgcagcggtcgggctgaacggggggttcgtgcacacagcccagcttggagcgaacgacctacaccgaactgagatacctacagcgtgagctatgagaaagcgccacgcttcccgaagggagaaaggcggacaggtatccggtaagcggcagggtcggaacaggagagcgcacgagggagcttccagggggaaacgcctggtatctttatagtcctgtcgggtttcgccacctctgacttgagcgtcgatttttgtgatgctcgtcaggggggcggagcctatggaaaaacgccagcaacgcggcctttttacggttcctggccttttgctggccttttgctcacatgttctttcctgcgttatcccctgattctgtggataaccgtattaccgcctttgagtgagctgataccgctcgccgcagccgaacgaccgagcgcagcgagtcagtgagcgaggaagcggaaga

SEQ ID NO: 16 - DNA, 36 bp, synthetic construct
  source 1..36: mol_type = other DNA
agttaaggagatatcatgacgcgctacgactccctg

SEQ ID NO: 17 - DNA, 36 bp, synthetic construct
  source 1..36: mol_type = other DNA
agcctttcgttttatttattccagcgcgtcctcggc

SEQ ID NO: 18 - DNA, 35 bp, synthetic construct
  source 1..35: mol_type = other DNA
ttacgccaagctagcccagcctgtttacgatgatc

SEQ ID NO: 19 - DNA, 36 bp, synthetic construct
  source 1..36: mol_type = other DNA
gtcgtagcgcgtcatgatatctccttaactgtatga

SEQ ID NO: 20 - DNA, 30 bp, synthetic construct
  source 1..30: mol_type = other DNA
gtgttgccgctggtggcttccaggatcgtg

SEQ ID NO: 21 - DNA, 30 bp, synthetic construct
  source 1..30: mol_type = other DNA
cacgatcctggaagccaccagcggcaacac

SEQ ID NO: 22 - DNA, 45 bp, synthetic construct
  source 1..45: mol_type = other DNA
gccctcgtcgatgttgcgcaggccgtacacgccctcgccgtaacg

SEQ ID NO: 23 - DNA, 45 bp, synthetic construct
  source 1..45: mol_type = other DNA
cgttacggcgagggcgtgtacggcctgcgcaacatcgacgagggc